European Patent Application EP 4 570 913 A1, published June 18, 2025. Title: ANTI-CGRP ANTIBODY AND USE. Applicant: Shanghai Junshi Biosciences Co., Ltd. The sequence listing filed with the application follows.

SEQUENCE LISTING (120 sequences)

SEQ ID NO: 1 - protein, 115 aa, synthetic construct
  source 1..115: note = 1F5HC VH
EVQLQQSGPELVKPGASVKISCKTSGYTFIDFNMHWVKQSHGKSLEWIGYIYPYNGDVVYNQNFTNKATLTVDSSSSTAYMELRRVTSEDSAIYYCAREGLGGYWGQGTTLTVSS

SEQ ID NO: 2 - protein, 5 aa, synthetic construct
  source 1..5: note = 1F5HC CDR1
DFNMH

SEQ ID NO: 3 - protein, 17 aa, synthetic construct
  source 1..17: note = 1F5HC CDR2-1
YIYPYNGDVVYNQNFTN

SEQ ID NO: 4 - protein, 6 aa, synthetic construct
  source 1..6: note = 1F5HC CDR3
EGLGGY

SEQ ID NO: 5 - protein, 115 aa, synthetic construct
  source 1..115: note = 1F5HC-1 VH
QVQLVQSGAEVKKPGASVKVSCKASGYTFIDFNMHWVRQAPGQRLEWMGYIYPYNGDVVYNQNFTNRVTLTVDTSSSTAYMELSSLRSEDTAVYYCAREGLGGYWGQGTLVTVSS

SEQ ID NO: 6 - protein, 115 aa, synthetic construct
  source 1..115: note = 1F5HC-2 VH
QVQLVQSGAEVKKPGASVKVSCKASGYTFTDFNMHWVRQAPGQRLEWMGYIYPYNGDVVYNQNFTNRVTLTVDTSSSTAYMELSSLRSEDTAVYYCAREGLGGYWGQGTLVTVSS

SEQ ID NO: 7 - protein, 115 aa, synthetic construct
  source 1..115: note = 1F5HC-3 VH
QVQLVQSGAEVKKPGASVKVSCKASGYTFTDFNMHWVRQAPGQGLEWMGYIYPYNGDVVYNQNFTNRVTLTVDTSSSTAYMELRSLRSDDTAVYYCAREGLGGYWGQGTLVTVSS

SEQ ID NO: 8 - protein, 115 aa, synthetic construct
  source 1..115: note = 1F5HC-4 VH
QVQLVQSGSELKKPGASVKVSCKASGYTFTDFNMHWVRQAPGQGLEWMGYIYPYNGDVVYNQNFTNRFVLSVDSSSSTAYLQISSLKAEDTAVYYCAREGLGGYWGQGTLVTVSS

SEQ ID NO: 9 - protein, 115 aa, synthetic construct
  source 1..115: note = 1F5HC-5 VH
QVQLVQSGAEVKKPGASVKVSCKASGYTFIDFNMHWVRQAPGQRLEWMGYIYPYNADVVYNQDFTNRVTLTVDTSSSTAYMELSSLRSEDTAVYYCAREGLGGYWGQGTLVTVSS

SEQ ID NO: 10 - protein, 115 aa, synthetic construct
  source 1..115: note = 3E5HC VH
EVQLQQSGPELVKPGASVKISCKTSGYTFTDYNMHWVKQSHGKSLEWIGYISPYNGGTAYNQKFKFKSTLTVDTSSSTAYMELRSLTSEDSAVYYCAREGLGGYWGQGTTLTVSS

SEQ ID NO: 11 - protein, 5 aa, synthetic construct
  source 1..5: note = 3E5HC CDR1
DYNMH

SEQ ID NO: 12 - protein, 17 aa, synthetic construct
  source 1..17: note = 3E5HC CDR2-1
YISPYNGGTAYNQKFKF

SEQ ID NO: 13 - protein, 6 aa, synthetic construct
  source 1..6: note = 3E5HC CDR3
EGLGGY

SEQ ID NO: 14 - protein, 115 aa, synthetic construct
  source 1..115: note = 3E5HC-1 VH
QVQLVQSGAEVKKPGASVKVSCKTSGYTFTDYNMHWVRQAPGQRLEWMGYISPYNGGTAYNQKFKFRVTLTVDTSSSTAYMELSSLRSEDTAVYYCAREGLGGYWGQGTLVTVSS

SEQ ID NO: 15 - protein, 115 aa, synthetic construct
  source 1..115: note = 3E5HC-2 VH
QVQLVQSGAEVKKPGASVKVSCKASGYTFTDYNMHWVRQAPGQRLEWMGYISPYNGGTAYNQKFKFRVTLTVDTSSSTAYMELSSLRSEDTAVYYCAREGLGGYWGQGTLVTVSS

SEQ ID NO: 16 - protein, 115 aa, synthetic construct
  source 1..115: note = 3E5HC-3 VH
QVQLVQSGAEVKKPGASVKVSCKASGYTFTDYNMHWVRQAPGQGLEWMGYISPYNGGTAYNQKFKFRVTLTVDTSSSTAYMELSRLRSDDTVVYYCAREGLGGYWGQGTLVTVSS

SEQ ID NO: 17 - protein, 115 aa, synthetic construct
  source 1..115: note = 3E5HC-4 VH
QVQLVQSGAEVKKPGASVKVSCKTSGYTFTDYNMHWVRQAPGQRLEWMGYISPYNAGTAYNQKFKFRVTLTVDTSSSTAYMELSSLRSEDTAVYYCAREGLGGYWGQGTLVTVSS

SEQ ID NO: 18 - protein, 115 aa, synthetic construct
  source 1..115: note = 2B8HC1 VH
EVQLQQSGPELVKPGASVKISCKASGYTFTDYNMHWVKQSHGKSLEWIGNIYPYNGGTVYNQKFNNKATLTVHTSSSTAYMDLRSLTSDDSAVYYCAREGLGGYWGQGTTLTVSS

SEQ ID NO: 19 - protein, 5 aa, synthetic construct
  source 1..5: note = 2B8HC1 CDR1
DYNMH

SEQ ID NO: 20 - protein, 17 aa, synthetic construct
  source 1..17: note = 2B8HC1 CDR2-1
NIYPYNGGTVYNQKFNN

SEQ ID NO: 21 - protein, 6 aa, synthetic construct
  source 1..6: note = 2B8HC1 CDR3
EGLGGY

SEQ ID NO: 22 - protein, 115 aa, synthetic construct
  source 1..115: note = 2B8HC1-1 VH
QVQLVQSGAEVKKPGASVKVSCKASGYTFTDYNMHWVRQAPGQGLEWMGNIYPYNGGTVYNQKFNNRVTLTVDTSSSTAYMELSRLRSDDTAVYYCAREGLGGYWGQGTLVTVSS

SEQ ID NO: 23 - protein, 115 aa, synthetic construct
  source 1..115: note = 2B8HC1-2 VH
QVQLVQSGAEVKKPGASVKVSCKASGYTFTDYNMHWVRQAPGQGLEWMGNIYPYNGGTVYNQKFNNRVTLTVDTSSSTAYMELRSLRSDDTAVYYCAREGLGGYWGQGTLVTVSS

SEQ ID NO: 24 - protein, 115 aa, synthetic construct
  source 1..115: note = 2B8HC1-3 VH
QVQLVQSGAEVKKPGASVKVSCKASGYTFTDYNMHWVRQAPGQGLEWMGNIYPYNAGTVYNQKFNNRVTLTVDTSSSTAYMELSRLRSDDTAVYYCAREGLGGYWGQGTLVTVSS

SEQ ID NO: 25 - protein, 115 aa, synthetic construct
  source 1..115: note = 2A2HC VH
EVQLQQSGPELVKPGASVKISCKASGYTFTDYNMHWVKQSHGKSLEWIGYVYPYNGGSAYNQKFKSKATLTVDTSSSIAYMDLHSLTSEDSAVYYCAREGLGGYWGQGTTLAVSS

SEQ ID NO: 26 - protein, 5 aa, synthetic construct
  source 1..5: note = 2A2HC CDR1
DYNMH

SEQ ID NO: 27 - protein, 17 aa, synthetic construct
  source 1..17: note = 2A2HC CDR2
YVYPYNGGSAYNQKFKS

SEQ ID NO: 28 - protein, 6 aa, synthetic construct
  source 1..6: note = 2A2HC CDR3
EGLGGY

SEQ ID NO: 29 - protein, 115 aa, synthetic construct
  source 1..115: note = 2A2HC-1 VH
QVQLVQSGAEVKKPGASVKVSCKASGYTFTDYNMHWVRQAPGQRLEWMGYVYPYNGGSAYNQKFKSRVTLTVDTSSSTAYMELSSLRSEDTAVYYCAREGLGGYWGQGTLVTVSS

SEQ ID NO: 30 - protein, 115 aa, synthetic construct
  source 1..115: note = 1B2HC VH
EVQLQQSGPEVVKPGASVRISCQASGYTFTDYNMHWVKQSHGKSLEWIGYIFPYNGVAVYNRKFRSKATLIIDKSSTTAYMELRSLTSEDSAVYYCAREGLGGYWGQGTTLTVSS

SEQ ID NO: 31 - protein, 5 aa, synthetic construct
  source 1..5: note = 1B2HC CDR1
DYNMH

SEQ ID NO: 32 - protein, 17 aa, synthetic construct
  source 1..17: note = 1B2HC CDR2
YIFPYNGVAVYNRKFRS

SEQ ID NO: 33 - protein, 6 aa, synthetic construct
  source 1..6: note = 1B2HC CDR3
EGLGGY

SEQ ID NO: 34 - protein, 115 aa, synthetic construct
  source 1..115: note = 1B2HC-1 VH
QVQLVQSGAEVKKPGASVKVSCKASGYTFTDYNMHWVRQAPGQGLEWMGYIFPYNGVAVYNRKFRSRVTLTIDTSSSTAYMELRSLRSDDTAVYYCAREGLGGYWGQGTLVTVSS

SEQ ID NO: 35 - protein, 115 aa, synthetic construct
  source 1..115: note = 1B2HC-2 VH
QVQLVQSGAEVKKPGASVKVSCKASGYTFTDYNMHWVRQAPGQRLEWMGYIFPYNGVAVYNRKFRSRVTLTVDTSSSTAYMELSSLRSEDTAVYYCAREGLGGYWGQGTLVTVSS

SEQ ID NO: 36 - protein, 115 aa, synthetic construct
  source 1..115: note = 3H10HC VH
EVQLQQSGPELVQPGASVKISCKASGYTFTDYNMHWVKQSHGESLEWIGYIYPYNGHTVYNQKFRNKATMTVDSSSSTAYMDLRSLTSEDSAVYYCAKEGLGGYWGQGTTLTVSS

SEQ ID NO: 37 - protein, 5 aa, synthetic construct
  source 1..5: note = 3H10HC CDR1
DYNMH

SEQ ID NO: 38 - protein, 17 aa, synthetic construct
  source 1..17: note = 3H10HC CDR2
YIYPYNGHTVYNQKFRN

SEQ ID NO: 39 - protein, 6 aa, synthetic construct
  source 1..6: note = 3H10HC CDR3
EGLGGY

SEQ ID NO: 40 - protein, 115 aa, synthetic construct
  source 1..115: note = 3H10HC-1 VH
QVQLVQSGAEVKKPGASVKVSCKASGYTFTDYNMHWVRQAPGQGLEWMGYIYPYNGHTVYNQKFRNRVTMTVDTSSSTAYMELRSLRSDDTAVYYCAKEGLGGYWGQGTLVTVSS

SEQ ID NO: 41 - protein, 115 aa, synthetic construct
  source 1..115: note = 3H10HC-2 VH
QVQLVQSGAEVKKPGASVKVSCKASGYTFTDYNMHWVRQAPGQGLEWMGYIYPYNGHTVYNQKFRNRVTLTVDTSSSTAYMELRSLRSDDTAVYYCAREGLGGYWGQGTLVTVSS

SEQ ID NO: 42 - protein, 117 aa, synthetic construct
  source 1..117: note = 3C1HC VH
EVQLQQSGPELVKPGASMKISCKASGYSFTGYTMNWVKQSHGNNLEWIGLINPYIGNTHYNQKFKDKATFTVDRSSSTAYMALLSLTSEDSAVYYCARELDSGFDYWGQGTTLTVSS

SEQ ID NO: 43 - protein, 5 aa, synthetic construct
  source 1..5: note = 3C1HC CDR1
GYTMN

SEQ ID NO: 44 - protein, 17 aa, synthetic construct
  source 1..17: note = 3C1HC CDR2
LINPYIGNTHYNQKFKD

SEQ ID NO: 45 - protein, 8 aa, synthetic construct
  source 1..8: note = 3C1HC CDR3
ELDSGFDY

SEQ ID NO: 46 - protein, 117 aa, synthetic construct
  source 1..117: note = 3C1HC-1 VH
QVQLVQSGAEVKKPGASVKVSCKASGYSFTGYTMNWVRQAPGQRLEWMGLINPYIGNTHYNQKFKDRVTFTVDRSSSTAYMELSSLRSEDTAVYYCARELDSGFDYWGQGTLVTVSS

SEQ ID NO: 47 - protein, 117 aa, synthetic construct
  source 1..117: note = 3C1HC-2 VH
QVQLVQSGAEVKKPGASVKVSCKASGYTFTGYTMNWVRQAPGQRLEWMGLINPYIGNTHYNQKFKDRVTFTVDRSSSTAYMELSSLRSEDTAVYYCARELDSGFDYWGQGTLVTVSS

SEQ ID NO: 48 - protein, 117 aa, synthetic construct
  source 1..117: note = 3C1HC-3 VH
QVQLVQSGSELKKPGASVKVSCKASGYTFTGYTMNWVRQAPGQGLEWMGLINPYIGNTHYNQKFKDRFVFSVDRSSSTAYLQISSLKAEDTAVYYCARELDSGFDYWGQGTLVTVSS

SEQ ID NO: 49 - protein, 117 aa, synthetic construct
  source 1..117: note = 3C1HC-4 VH
QVQLVQSGAEVKKPGASVKVSCKASGYTFTGYTMNWVRQAPGQGLEWMGLINPYIGNTHYNQKFKDRVTFTVDRSSSTAYMELSRLRSDDTAVYYCARELDSGFDYWGQGTLVTVSS

SEQ ID NO: 50 - protein, 111 aa, synthetic construct
  source 1..111: note = 1A2LC2 VL
DIVLTQSPASLAVSLGQRATISCKASQNIDYDGYAYLNWYQQKPGQPPKVLIYSVFNLESGIPARFSGSGSGTDFTLNIHPVEEEDAATYYCQQSNEFPYTFGGGTKLEVK

SEQ ID NO: 51 - protein, 15 aa, synthetic construct
  source 1..15: note = 1A2LC2 CDR1
KASQNIDYDGYAYLN

SEQ ID NO: 52 - protein, 7 aa, synthetic construct
  source 1..7: note = 1A2LC2 CDR2
SVFNLES

SEQ ID NO: 53 - protein, 9 aa, synthetic construct
  source 1..9: note = 1A2LC2 CDR3
QQSNEFPYT

SEQ ID NO: 54 - protein, 111 aa, synthetic construct
  source 1..111: note = 1A2LC2-1 VL
DIVLTQSPASLAVSPGQRATITCKASQNIDYDGYAYLNWYQQKPGQPPKVLIYSVFNLESGVPARFSGSGSGTDFTLTINPVEANDTANYYCQQSNEFPYTFGQGTKLEIK

SEQ ID NO: 55 - protein, 111 aa, synthetic construct
  source 1..111: note = 1A2LC2-2 VL
DIVLTQSPASLAVSPGQRATITCKASQNIDYDGYAYLNWYQQKPGQPPKVLIYSVFNLESGVPARFSGSGSGTDFTLTINPVEADDTANYYCQQSNEFPYTFGQGTKLEIK

SEQ ID NO: 56 - protein, 111 aa, synthetic construct
  source 1..111: note = 1A2LC2-3 VL
EIVLTQSPATLSLSPGERATLSCKASQNIDYDGYAYLNWYQQKPGQAPRVLIYSVFNLESGIPARFSGSGSGTDFTLTISSLEPEDFAVYYCQQSNEFPYTFGQGTKLEIK

SEQ ID NO: 57 - protein, 111 aa, synthetic construct
  source 1..111: note = 1A2LC2-4 VL
DIQLTQSPSFLSASVGDRVTITCKASQNIDYDGYAYLNWYQQKPGKAPKVLIYSVFNLESGVPSRFSGSGSGTEFTLTISSLQPEDFATYYCQQSNEFPYTFGQGTKLEIK

SEQ ID NO: 58 - protein, 111 aa, synthetic construct
  source 1..111: note = 1F5LC1 VL
DIVLTQSPASLAVSLGQRATISCKASQNIDFDGYAYMNWYQHKPGQPPRVLIYSVFNLESGIPARFSGSGSGTDFTLNIHPVEEEDAATYYCQQSHEVPYTFGGGTNLEIK

SEQ ID NO: 59 - protein, 15 aa, synthetic construct
  source 1..15: note = 1F5LC1 CDR1
KASQNIDFDGYAYMN

SEQ ID NO: 60 - protein, 7 aa, synthetic construct
  source 1..7: note = 1F5LC1 CDR2
SVFNLES

SEQ ID NO: 61 - protein, 9 aa, synthetic construct
  source 1..9: note = 1F5LC1 CDR3
QQSHEVPYT

SEQ ID NO: 62 - protein, 111 aa, synthetic construct
  source 1..111: note = 1F5LC1-1 VL
EIVLTQSPATLSLSPGERATLSCKASQNIDFDGYAYMNWYQQKPGQAPRVLIYSVFNLESGIPARFSGSGSGTDFTLTISSLEPEDFAVYYCQQSHEVPYTFGQGTKLEIK

SEQ ID NO: 63 - protein, 111 aa, synthetic construct
  source 1..111: note = 1F5LC1-2 VL
EIVLTQSPATLSLSPGERATLSCKASQNIDFDGYAYMNWYQHKPGQAPRVLIYSVFNLESGIPARFSGSGSGTDFTLTISSLEPEDFAVYYCQQSHEVPYTFGQGTKLEIK

SEQ ID NO: 64 - protein, 111 aa, synthetic construct
  source 1..111: note = 1F5LC1-3 VL
DIVLTQSPASLAVSPGQRATITCKASQNIDFDGYAYMNWYQQKPGQPPKVLIYSVFNLESGVPARFSGSGSGTDFTLTINPVEADDTANYYCQQSHEVPYTFGQGTKLEIK

SEQ ID NO: 65 - protein, 111 aa, synthetic construct
  source 1..111: note = 1F5LC1-4 VL
DIVLTQSPDSLAVSLGERATINCKASQNIDFDGYAYMNWYQHKPGQPPKVLIYSVFNLESGVPDRFSGSGSGTDFTLTISSLQAEDVAVYYCQQSHEVPYTFGQGTKLEIK

SEQ ID NO: 66 - protein, 109 aa, synthetic construct
  source 1..109: note = 2B8LC2 VL
DVVLTQSPTSLAVSLGQRATISCQASQNIDGNTYMNWYQQKPGQPPKVLIYSIFNLESGIPARFSGSGSGTHFTLTIHPVEEEDAATYYCQQSNDYPYTFGGGTKLEIK

SEQ ID NO: 67 - protein, 13 aa, synthetic construct
  source 1..13: note = 2B8LC2 CDR1
QASQNIDGNTYMN

SEQ ID NO: 68 - protein, 7 aa, synthetic construct
  source 1..7: note = 2B8LC2 CDR2
SIFNLES

SEQ ID NO: 69 - protein, 9 aa, synthetic construct
  source 1..9: note = 2B8LC2 CDR3
QQSNDYPYT

SEQ ID NO: 70 - protein, 109 aa, synthetic construct
  source 1..109: note = 2B8LC2-1 VL
DIVLTQSPDSLAVSLGERATINCQASQNIDGNTYMNWYQQKPGQPPKVLIYSIFNLESGVPDRFSGSGSGTDFTLTISSLQAEDVAVYYCQQSNDYPYTFGQGTKLEIK

SEQ ID NO: 71 - protein, 109 aa, synthetic construct
  source 1..109: note = 2B8LC2-2 VL
DVQLTQSPSFLSASVGDRVTITCQASQNIDGNTYMNWYQQKPGKAPKVLIYSIFNLESGVPSRFSGSGSGTEFTLTISSLQPEDFATYYCQQSNDYPYTFGQGTKLEIK

SEQ ID NO: 72 - protein, 112 aa, synthetic construct
  source 1..112: note = 3C1LC VL
DVLMTQTPLSLPVSLGDQASLSCRSSQNIVHSNGDTYLEWYLQKPGQSPKLLIYKVSNRFSGVPDRFSGSGSGTDFTLKISRVEAEDLGVYYCYQGSHVPWTFGGGTKLEIK

SEQ ID NO: 73 - protein, 16 aa, synthetic construct
  source 1..16: note = 3C1LC CDR1-1
RSSQNIVHSNGDTYLE

SEQ ID NO: 74 - protein, 7 aa, synthetic construct
  source 1..7: note = 3C1LC CDR2
KVSNRFS

SEQ ID NO: 75 - protein, 9 aa, synthetic construct
  source 1..9: note = 3C1LC CDR3
YQGSHVPWT

SEQ ID NO: 76 - protein, 112 aa, synthetic construct
  source 1..112: note = 3C1LC-1 VL
DVVMTQSPLSLPVTLGQPASISCRSSQNIVHSNGDTYLEWYQQRPGQSPRLLIYKVSNRFSGVPDRFSGSGSGTDFTLKISRVEAEDVGVYYCYQGSHVPWTFGQGTKLEIK

SEQ ID NO: 77 - protein, 112 aa, synthetic construct
  source 1..112: note = 3C1LC-2 VL
DVVMTQTPLSLSVTPGQPASISCRSSQNIVHSNGDTYLEWYLQKPGQSPQLLIYKVSNRFSGVPDRFSGSGSGTDFTLKISRVEAEDVGVYYCYQGSHVPWTFGQGTKLEIK

SEQ ID NO: 78 - protein, 112 aa, synthetic construct
  source 1..112: note = 3C1LC-3 VL
DVVMTQSPDSLAVSLGERATINCRSSQNIVHSNGDTYLEWYQQKPGQPPKLLIYKVSNRFSGVPDRFSGSGSGTDFTLTISSLQAEDVAVYYCYQGSHVPWTFGQGTKLEIK

SEQ ID NO: 79 - protein, 112 aa, synthetic construct
  source 1..112: note = 3C1LC-4 VL
DVVMTQSPDSLAVSLGERATINCRSSQNIVHSNADTYLEWYQQKPGQPPKLLIYKVSNRFSGVPDRFSGSGSGTDFTLTISSLQAEDVAVYYCYQGSHVPWTFGQGTKLEIK

SEQ ID NO: 80 - protein, 111 aa, synthetic construct
  source 1..111: note = 3E5LC VL
DIVLTQSPASLAVSLGQRATISCKASQNIDYDGYTYLNWYQQKPGQPPKVLIYSIFNLESGIPARFSGSGSGTDFTLNIHPVEEEDAATYYCQQSNEVPYTFGGGTKLEIK

SEQ ID NO: 81 - protein, 15 aa, synthetic construct
  source 1..15: note = 3E5LC CDR1
KASQNIDYDGYTYLN

SEQ ID NO: 82 - protein, 7 aa, synthetic construct
  source 1..7: note = 3E5LC CDR2
SIFNLES

SEQ ID NO: 83 - protein, 9 aa, synthetic construct
  source 1..9: note = 3E5LC CDR3
QQSNEVPYT

SEQ ID NO: 84 - protein, 111 aa, synthetic construct
  source 1..111: note = 3E5LC-1 VL
DIVLTQSPDSLAVSLGERATINCKASQNIDYDGYTYLNWYQQKPGQPPKVLIYSIFNLESGVPDRFSGSGSGTDFTLTISSLQAEDVAVYYCQQSNEVPYTFGQGTKLEIK

SEQ ID NO: 85 - protein, 111 aa, synthetic construct
  source 1..111: note = 3H10LC2 VL
DIVLTQSPDSLAVSLGQRATISCKASQNIDYGGYSYMNWYQQKPGQPPKVLIYSVFNLESGIPARFSGSGSGTDFTLTIHPVEEEDAATYYCQQSNEAPYTFGGGTKLEIR

SEQ ID NO: 86 - protein, 15 aa, synthetic construct
  source 1..15: note = 3H10LC2 CDR1
KASQNIDYGGYSYMN

SEQ ID NO: 87 - protein, 7 aa, synthetic construct
  source 1..7: note = 3H10LC2 CDR2
SVFNLES

SEQ ID NO: 88 - protein, 9 aa, synthetic construct
  source 1..9: note = 3H10LC2 CDR3
QQSNEAPYT

SEQ ID NO: 89 - protein, 111 aa, synthetic construct
  source 1..111: note = 3H10LC2-1 VL
DIVLTQSPDSLAVSLGERATINCKASQNIDYGGYSYMNWYQQKPGQPPKVLIYSVFNLESGVPDRFSGSGSGTDFTLTISSLQAEDVAVYYCQQSNEAPYTFGQGTKLEIK

SEQ ID NO: 90 - protein, 111 aa, synthetic construct
  source 1..111: note = 3H10LC2-2 VL
DIQLTQSPSSLSASVGDRVTITCKASQNIDYGGYSYMNWYQQKPGKAPKVLIYSVFNLESGVPSRFSGSGSGTDFTLTISSLQPEDFATYYCQQSNEAPYTFGQGTKLEIK

SEQ ID NO: 91 - protein, 219 aa, synthetic construct
  source 1..219: note = Hu224 LC
DVVMTQSPDSLAVSLGERATINCRSSQNIVHSNGDTYLEWYQQKPGQPPKLLIYKVSNRFSGVPDRFSGSGSGTDFTLTISSLQAEDVAVYYCYQGSHVPWTFGQGTKLEIKRTVAAPSVFIFPPSDEQLKSGTASVVCLLNNFYPREAKVQWKVDNALQSGNSQESVTEQDSKDSTYSLSSTLTLSKADYEKHKVYACEVTHQGLSSPVTKSFNRGEC

SEQ ID NO: 92 - protein, 444 aa, synthetic construct
  source 1..444: note = Hu224 HC
QVQLVQSGAEVKKPGASVKVSCKASGYSFTGYTMNWVRQAPGQRLEWMGLINPYIGNTHYNQKFKDRVTFTVDRSSSTAYMELSSLRSEDTAVYYCARELDSGFDYWGQGTLVTVSSASTKGPSVFPLAPCSRSTSESTAALGCLVKDYFPEPVTVSWNSGALTSGVHTFPAVLQSSGLYSLSSVVTVPSSSLGTKTYTCNVDHKPSNTKVDKRVESKYGPPCPPCPAPEFLGGPSVFLFPPKPKDTLMISRTPEVTCVVVDVSQEDPEVQFNWYVDGVEVHNAKTKPREEQFNSTYRVVSVLTVLHQDWLNGKEYKCKVSNKGLPSSIEKTISKAKGQPREPQVYTLPPSQEEMTKNQVSLTCLVKGFYPSDIAVEWESNGQPENNYKTTPPVLDSDGSFFLYSRLTVDKSRWQEGNVFSCSVMHEALHNHYTQKSLSLSLGK

SEQ ID NO: 93 - protein, 219 aa, synthetic construct; identical to SEQ ID NO: 91
  source 1..219: note = Hu228LC

SEQ ID NO: 94 - protein, 444 aa, synthetic construct
  source 1..444: note = Hu228HC
QVQLVQSGAEVKKPGASVKVSCKASGYTFTGYTMNWVRQAPGQRLEWMGLINPYIGNTHYNQKFKDRVTFTVDRSSSTAYMELSSLRSEDTAVYYCARELDSGFDYWGQGTLVTVSSASTKGPSVFPLAPCSRSTSESTAALGCLVKDYFPEPVTVSWNSGALTSGVHTFPAVLQSSGLYSLSSVVTVPSSSLGTKTYTCNVDHKPSNTKVDKRVESKYGPPCPPCPAPEFLGGPSVFLFPPKPKDTLMISRTPEVTCVVVDVSQEDPEVQFNWYVDGVEVHNAKTKPREEQFNSTYRVVSVLTVLHQDWLNGKEYKCKVSNKGLPSSIEKTISKAKGQPREPQVYTLPPSQEEMTKNQVSLTCLVKGFYPSDIAVEWESNGQPENNYKTTPPVLDSDGSFFLYSRLTVDKSRWQEGNVFSCSVMHEALHNHYTQKSLSLSLGK

SEQ ID NO: 95 - protein, 219 aa, synthetic construct
  source 1..219: note = Hu231LC
DVVMTQTPLSLSVTPGQPASISCRSSQNIVHSNGDTYLEWYLQKPGQSPQLLIYKVSNRFSGVPDRFSGSGSGTDFTLKISRVEAEDVGVYYCYQGSHVPWTFGQGTKLEIKRTVAAPSVFIFPPSDEQLKSGTASVVCLLNNFYPREAKVQWKVDNALQSGNSQESVTEQDSKDSTYSLSSTLTLSKADYEKHKVYACEVTHQGLSSPVTKSFNRGEC

SEQ ID NO: 96 - protein, 444 aa, synthetic construct
  source 1..444: note = Hu231HC
QVQLVQSGSELKKPGASVKVSCKASGYTFTGYTMNWVRQAPGQGLEWMGLINPYIGNTHYNQKFKDRFVFSVDRSSSTAYLQISSLKAEDTAVYYCARELDSGFDYWGQGTLVTVSSASTKGPSVFPLAPCSRSTSESTAALGCLVKDYFPEPVTVSWNSGALTSGVHTFPAVLQSSGLYSLSSVVTVPSSSLGTKTYTCNVDHKPSNTKVDKRVESKYGPPCPPCPAPEFLGGPSVFLFPPKPKDTLMISRTPEVTCVVVDVSQEDPEVQFNWYVDGVEVHNAKTKPREEQFNSTYRVVSVLTVLHQDWLNGKEYKCKVSNKGLPSSIEKTISKAKGQPREPQVYTLPPSQEEMTKNQVSLTCLVKGFYPSDIAVEWESNGQPENNYKTTPPVLDSDGSFFLYSRLTVDKSRWQEGNVFSCSVMHEALHNHYTQKSLSLSLGK

SEQ ID NO: 97 - protein, 37 aa, synthetic construct
  source 1..37: note = CGRP 1-37 (WT)
ACDTATCVTHRLAGLLSRSGGVVKNNFVPTNVGSKAF

SEQ ID NO: 98 - protein, 13 aa, synthetic construct
  source 1..13: note = CGRP 1-13
ACDTATCVTHRLA

SEQ ID NO: 99 - protein, 19 aa, synthetic construct
  source 1..19: note = CGRP 1-19
ACDTATCVTHRLAGLLSRS

SEQ ID NO: 100 - protein, 12 aa, synthetic construct
  source 1..12: note = CGRP 8-19
VTHRLAGLLSRS

SEQ ID NO: 101 - protein, 19 aa, synthetic construct
  source 1..19: note = CGRP 8-26
VTHRLAGLLSRSGGVVKNN

SEQ ID NO: 102 - protein, 12 aa, synthetic construct
  source 1..12: note = CGRP 13-24
AGLLSRSGGVVK

SEQ ID NO: 103 - protein, 5 aa, synthetic construct
  source 1..5: note = HCDR1
  VARIANT 2: note; note (original language) = X is F or Y
DXNMH

SEQ ID NO: 104 - protein, 17 aa, synthetic construct
  source 1..17: note = HCDR2
  VARIANT 1: note; note (original language) = X is Y or N
  VARIANT 2: note; note (original language) = X is I or V
  VARIANT 3: note; note (original language) = X is Y, S, or F
  VARIANT 7: note; note (original language) = X is G or A
  VARIANT 8: note; note (original language) = X is D, G, V, or H
  VARIANT 9: note; note (original language) = X is V, T, S, or A
  VARIANT 10: note; note (original language) = X is V or A
  VARIANT 13: note; note (original language) = X is Q or R
  VARIANT 14: note; note (original language) = X is K or N
  VARIANT 16: note; note (original language) = X is T, K, N, or R
  VARIANT 17: note; note (original language) = X is N, F, or S
XXXPYNXXXXYNXXFXX

SEQ ID NO: 105 - protein, 10 aa, synthetic construct
  source 1..10: note = LCDR1
  VARIANT 1: note; note (original language) = X13 is K, Q, or R
  VARIANT 2: note; note (original language) = X is A or S
  VARIANT 7: note; note (original language) = X is SEQ ID NO: 114, SEQ ID NO: 115, SEQ ID NO: 116, SEQ ID NO: 117, SEQ ID NO: 118, SEQ ID NO: 119, or SEQ ID NO: 120
  VARIANT 9: note; note (original language) = X is L or M
  VARIANT 10: note; note (original language) = X is N or E
XXSQNIXYXX

SEQ ID NO: 106 - protein, 7 aa, synthetic construct
  source 1..7: note = LCDR2
  VARIANT 2: note; note (original language) = X is V or I
SXFNLES

SEQ ID NO: 107 - protein, 9 aa, synthetic construct
  source 1..9: note = LCDR3
  VARIANT 1: note; note (original language) = X is Q
  VARIANT 4: note; note (original language) = X is N or H
  VARIANT 5: note; note (original language) = X is E or D
  VARIANT 6: note; note (original language) = X is F, V, Y, or A
XQSXXXPYT

SEQ ID NO: 108 - protein, 327 aa, synthetic construct
  source 1..327: note; note (original language) = Heavy chain constant region
ASTKGPSVFPLAPCSRSTSESTAALGCLVKDYFPEPVTVSWNSGALTSGVHTFPAVLQSSGLYSLSSVVTVPSSSLGTKTYTCNVDHKPSNTKVDKRVESKYGPPCPPCPAPEFLGGPSVFLFPPKPKDTLMISRTPEVTCVVVDVSQEDPEVQFNWYVDGVEVHNAKTKPREEQFNSTYRVVSVLTVLHQDWLNGKEYKCKVSNKGLPSSIEKTISKAKGQPREPQVYTLPPSQEEMTKNQVSLTCLVKGFYPSDIAVEWESNGQPENNYKTTPPVLDSDGSFFLYSRLTVDKSRWQEGNVFSCSVMHEALHNHYTQKSLSLSLGK

SEQ ID NO: 109 - protein, 107 aa, synthetic construct [sequence omitted]

SEQ ID NO: 110 - protein, 17 aa, synthetic construct
  source 1..17: note = 1F5HC CDR2-2
YIYPYNADVVYNQDFTN

SEQ ID NO: 111 - protein, 17 aa, synthetic construct
  source 1..17: note = 3E5HC CDR2-2
YISPYNAGTAYNQKFKF

SEQ ID NO: 112 - protein, 17 aa, synthetic construct
  source 1..17: note = 2B8HC1 CDR2-2
NIYPYNAGTVYNQKFNN

SEQ ID NO: 113 - protein, 16 aa, synthetic construct
  source 1..16: note = 3C1LC CDR1-2
RSSQNIVHSNADTYLE

SEQ ID NO: 114 - protein, 6 aa, synthetic construct
  source 1..6: note; note (original language) = Z in SEQ ID NO: 105
DYDGYA

SEQ ID NO: 115 - protein, 6 aa, synthetic construct
  source 1..6: note; note (original language) = Z in SEQ ID NO: 105
DFDGYA

SEQ ID NO: 116 - protein, 4 aa, synthetic construct
  source 1..4: note; note (original language) = Z in SEQ ID NO: 105
DGNT

SEQ ID NO: 117 - protein, 7 aa, synthetic construct
  source 1..7: note; note (original language) = Z in SEQ ID NO: 105
VHSNGDT

SEQ ID NO: 118 - protein, 7 aa, synthetic construct
  source 1..7: note; note (original language) = Z in SEQ ID NO: 105
VHSNADT

SEQ ID NO: 119 - protein, 6 aa, synthetic construct
  source 1..6: note; note (original language) = Z in SEQ ID NO: 105
DYDGYT

SEQ ID NO: 120 - protein, 6 aa, synthetic construct
  source 1..6: note; note (original language) = Z in SEQ ID NO: 105
DYGGYS